European Patent Application EP 4 810 517 A1, published September 23, 2026. Title: Antigen binding proteins specifically binding MAGE-A4. Applicant: BioCopy AG. Application EP. The sequence listing filed with the application follows.

SEQUENCE LISTING (63 sequences)

SEQ ID NO: 1 - protein, 10 aa, Homo sapiens
GVYDGREHTV

SEQ ID NO: 2 - protein, 6 aa, synthetic construct
SNKWWN

SEQ ID NO: 3 - protein, 16 aa, synthetic construct
EVYHSGSTNYNPSLKS

SEQ ID NO: 4 - protein, 9 aa, synthetic construct
DYSNYGFDY

SEQ ID NO: 5 - protein, 11 aa, synthetic construct
QASQDINNYLN

SEQ ID NO: 6 - protein, 7 aa, synthetic construct
DASNLET

SEQ ID NO: 7 - protein, 11 aa, synthetic construct
QQYDNLPRSIT

SEQ ID NO: 8 - protein, 5 aa, synthetic construct
SYSMN

SEQ ID NO: 9 - protein, 17 aa, synthetic construct
SISSRSSFMYYADSVKG

SEQ ID NO: 10 - protein, 10 aa, synthetic construct
ETWNYGAFDI

SEQ ID NO: 11 - protein, 12 aa, synthetic construct
RASQSVSSSYLA

SEQ ID NO: 12 - protein, 7 aa, synthetic construct
GASSRAT

SEQ ID NO: 13 - protein, 10 aa, synthetic construct
QQYGTSPALT

SEQ ID NO: 14 - protein, 118 aa, synthetic construct
QVQLVQSGPGLVKPSGTLSLTCAVSGVSISSNKWWNWVRQPPGKGLEWIGEVYHSGSTNYNPSLKSRVTISVDKSKNQFSLRLSSVTAADTAVYYCARDYSNYGFDYWGQGALVTVSS

SEQ ID NO: 15 - protein, 109 aa, synthetic construct
DIVMTQSPSSLSASVGDRVTITCQASQDINNYLNWYQQKPGKAPKLLIYDASNLETGVPSRFSGSGSGTDFTFTISSLQPEDIATYFCQQYDNLPRSITFGQGTRLEIK

SEQ ID NO: 16 - protein, 119 aa, synthetic construct
QVQLQESGGGLVKPGGSLRLSCAASGFTFSSYSMNWVRQAPGRGLEWVSSISSRSSFMYYADSVKGRFTISRDNAKNSLYLQMSSLRAEDTAVFYCARETWNYGAFDIWGQGTMVTVSS

SEQ ID NO: 17 - protein, 109 aa, synthetic construct
EIVLTQSPGTLSLSPGERATLSCRASQSVSSSYLAWYQQKPGQAPRLLIYGASSRATGIPDRFSGSGSGTDFTLTISRLEPEDFAVYYCQQYGTSPALTFGGGTKVEIK

SEQ ID NO: 18 - protein, 10 aa, Homo sapiens
GLYDGREHSV

SEQ ID NO: 19 - protein, 10 aa, Homo sapiens
GVYDGEEHSV

SEQ ID NO: 20 - protein, 10 aa, Homo sapiens
GIYDGKRHLI

SEQ ID NO: 21 - protein, 10 aa, Homo sapiens
GIYDGILHSI

SEQ ID NO: 22 - protein, 10 aa, synthetic construct
XXYDGRXHXX

SEQ ID NO: 23 - protein, 317 aa, Homo sapiens
MSSEQKSQHCKPEEGVEAQEEALGLVGAQAPTTEEQEAAVSSSSPLVPGTLEEVPAAESAGPPQSPQGASALPTTISFTCWRQPNEGSSSQEEEGPSTSPDAESLFREALSNKVDELAHFLLRKYRAKELVTKAEMLERVIKNYKRCFPVIFGKASESLKMIFGIDVKEVDPASNTYTLVTCLGLSYDGLLGNNQIFPKTGLLIIVLGTIAMEGDSASEEEIWEELGVMGVYDGREHTVYGEPRKLLTQDWVQENYLEYRQVPGSNPARYEFLWGPRALAETSYVKVLEHVVRVNARVRIAYPSLREAALLEEEEGV

SEQ ID NO: 24 - protein, 315 aa, Mus musculus
MENPDNTHYCSLQGSARSQRELDNVQATIAVVDEEEATPTSKKVYSSGLPSPPQSPQRASSPLVILASVPEGPSEEASTNQVEEQEDPLCMLYNAQNIKLYELATFLFFKYQMKAFTTKAEMLESIGREYEEYYPLIFSEASECFKLVSGIGMIEVDPFVQSYILVPALGLTYDGMLTDVQSKPKTGILIVVLGAIFTQGNCVSEEIIWKMLNNIGLYGGRHLYIHQDPRKFISEEFVHEGYLEYRQVPNSDPPSYEFLWDPRAFAETTKMKVLEIFASITMTDPRAYTEKYAEALRDETERAQARIIQQIVLQL

SEQ ID NO: 25 - protein, 5 aa, synthetic construct
GGGGS

SEQ ID NO: 26 - protein, 10 aa, synthetic construct
GGGGSGGGGS

SEQ ID NO: 27 - protein, 15 aa, synthetic construct
GGGGSGGGGSGGGGS

SEQ ID NO: 28 - protein, 5 aa, synthetic construct
GGGSG

SEQ ID NO: 29 - protein, 5 aa, synthetic construct
GGSGG

SEQ ID NO: 30 - protein, 5 aa, synthetic construct
GSGGG

SEQ ID NO: 31 - protein, 6 aa, synthetic construct
GSGGGP

SEQ ID NO: 32 - protein, 5 aa, synthetic construct
GGEPS

SEQ ID NO: 33 - protein, 7 aa, synthetic construct
GGEGGGP

SEQ ID NO: 34 - protein, 12 aa, synthetic construct
GGEGGGSEGGGS

SEQ ID NO: 35 - protein, 8 aa, synthetic construct
GGGSGGGG

SEQ ID NO: 36 - protein, 24 aa, synthetic construct
GGGGSGGGGSGGGGSGGGGSGGGS

SEQ ID NO: 37 - protein, 20 aa, synthetic construct
GGGGSGGGGSGGGGSGGGGS

SEQ ID NO: 38 - protein, 15 aa, synthetic construct
EAAAKEAAAKEAAAK

SEQ ID NO: 39 - protein, 10 aa, Homo sapiens
GLADGRTHTV

SEQ ID NO: 40 - protein, 10 aa, Homo sapiens
GLYDGPVHEV

SEQ ID NO: 41 - protein, 10 aa, synthetic construct
AVYDGREHTV

SEQ ID NO: 42 - protein, 10 aa, synthetic construct
GAYDGREHTV

SEQ ID NO: 43 - protein, 10 aa, synthetic construct
GVADGREHTV

SEQ ID NO: 44 - protein, 10 aa, synthetic construct
GVYAGREHTV

SEQ ID NO: 45 - protein, 10 aa, synthetic construct
GVYDAREHTV

SEQ ID NO: 46 - protein, 10 aa, synthetic construct
GVYDGAEHTV

SEQ ID NO: 47 - protein, 10 aa, synthetic construct
GVYDGRAHTV

SEQ ID NO: 48 - protein, 10 aa, synthetic construct
GVYDGREATV

SEQ ID NO: 49 - protein, 10 aa, synthetic construct
GVYDGREHAV

SEQ ID NO: 50 - protein, 10 aa, synthetic construct
GVYDGREHTA

SEQ ID NO: 51 - protein, 10 aa, Homo sapiens
EVYDGREHSA

SEQ ID NO: 52 - protein, 10 aa, Homo sapiens
EVFEGREDSV

SEQ ID NO: 53 - protein, 10 aa, Homo sapiens
EVFEGREDSI

SEQ ID NO: 54 - protein, 10 aa, Homo sapiens
GLYDGREHSV

SEQ ID NO: 55 - protein, 10 aa, Homo sapiens
GVYVGKEHMF

SEQ ID NO: 56 - protein, 10 aa, Homo sapiens
GLYDGMEHLI

SEQ ID NO: 57 - protein, 10 aa, Homo sapiens
GVYAGREHFL

SEQ ID NO: 58 - protein, 10 aa, Homo sapiens
EASDGREDSV

SEQ ID NO: 59 - protein, 10 aa, Homo sapiens
GVYDGEEHSV

SEQ ID NO: 60 - protein, 10 aa, Homo sapiens
GIYDGKRHLI

SEQ ID NO: 61 - protein, 10 aa, Homo sapiens
GIYDGILHSI

SEQ ID NO: 62 - protein, 10 aa, Homo sapiens
GLYDGIEHFM

SEQ ID NO: 63 - protein, 10 aa, Homo sapiens
GVYAGREHFV